European Patent Application EP 4 227 409 A1, published August 16, 2023. Title: Target sequence-specific alteration technique using CRISPR type I-D system. Applicant: Tokushima University. The sequence listing filed with the application follows.

SEQUENCE LISTING (42 sequences)

SEQ ID NO: 1 - protein, 721 aa, Microcystis aeruginosa
MGNYQVTLKPVYSCPADEIPDGIKVPQGWRLSWHQVETWKALNDPDIDVIFNTAMTGDGKSLAAYLRTLQGYFPIMGLYPTNELARDQRGQIEAYIQRFQPTDQPRVNLLTGPELELYAERDGKTKAIALETRSKQSEILLTNPDIFHYLHRAAYLTPYDNPDQLWNRIDKHFDLFLFDEFHVFGTPQVASIINTMLLIRRANRGKRYLFLSATPDEGLLKRLDKAGFRYRSIDPVREGKYRFPDTPEEANSLAQQGWRQVTSEIELSFIPLPSSFQTSENWLKENKERILDYFKRYPGSKGAIILNSIASVKRLLPIFRELLATIGLTVGENTGLSGTREKLASLNRDLVIGTSTIDVGVDFKINFLIFESSDAGNFIQRFGRLGRHSGYDRKGTAVKFTNFTAIALVPKFFLERLFEKKDAPLQVGERYDRIQLQEAIKSNYRHINNFEGYYQRWGAVQSFQLWWNLGSPKIKSQYGESRQKFQQECEEVFDTSLKRVAGRVKGWADEWKELSGKNGNPIFEDASSFRGSSPLLCGLYDSTEPEECDRFKTYDLPSILGNLEVEVWRKGEFKRQIEATKTPIARRRFDYCLAFLNLKGYREERLNWRFTYDGDLGEIASAWKVQVLTGIGVWQPDNPWLDRISRELRDLALVSFVFAYPVAAVRQRLQLPMHFGIYPISDESSLHSPLSPYSIAIGQAALLLDTLAHRFKGKGGEVWIC

SEQ ID NO: 2 - protein, 224 aa, Microcystis aeruginosa
MVHIYSCQLELHDSLYYATREIGRLYESEPVIHNYALCYALGLVNSDSYRYFCSEQIPQYQEHLNPLNEEKIYVTPARAIAHTAVLNTWKYANNNYHVEMEKTQKNIPSFGRAKEIAPESIFECFIISHHPLQLPKWIRLGKWMSKAEVKLTELSLSKQKEDLFIYPYPLNPLDVMFTHQVIGYDVINMPPVSLIRNVRMRGEYYQISDRPDLKIPARLSYHFG

SEQ ID NO: 3 - protein, 277 aa, Microcystis aeruginosa
MPYSLVLNLTPRSPIYPNFLTGRHLHALFLTLVSSVDQELGNILHTAEADKAFTLSPLQMQSGGKTINSPQWRHEREIASETPCWWRISLLDDRLFGKLTSLWLNLNPKQPWHLGSADLVITSVLATPQSVQPWANSCTYQYLYENASETNREFDFLFATPVTFRQGKFDSALPTRELVFNSLLGRWNRYSGIPFDSIALESIFPSFFDIQTKLADEAYKNQSIGCVGEIHYRLLGEVEPAKIKAINALADFALYAGVGRKTTMGMGMTRRISKDKR

SEQ ID NO: 4 - protein, 332 aa, Microcystis aeruginosa
TFLTSVDAKFFHSEIPYKPMGKYVHFLTIRVTESYPLFQTDGELNKARVRAGIDSKKTISRLSMFKRKQSTPERLVGRELLRNYGLITAEECEYNVKFAMNNADCIIYGFAIGDSGSEKSKVVVDTAFSITPFDESHESFTLNAPYENGTMASKGENNTKVGEVTSRINQQDHIRPQVFFPSIVTLKDPTEASFLYVFNNILRTRHYGAQTTRTGRVRNELIGVIFADGEIVSNLRWTQAIYDRLPDEVLHSIDPLDEDLVMEKATEAIQALMAEEFIVHTDFIGENFQPLLTEVKTLTGTEAGILSVLDQANKESKKYFEQYIEKKKAEKK

SEQ ID NO: 5 - protein, 1156 aa, Microcystis aeruginosa
MPKKQKKLEETGQLNLFDNTTEIDDEDLDFEFEDIDLESLVSEDLGITESVSDRRVETVRQLLTLKLLREAIRAENPDDRVMADFAEMVLPNLLRLAIGVTAKGGNFIEAVDRGRELRNKPKAKRDNAGDQSLNTHLLNGLFPANLIEKRLQKLNTTVRRIIKEFERRLAIAGFLVHDFEKFSYDRFPSMSERYIQIQRDFIQDPFKNQDPRKLSREEHREILQVLIPELGLDRFLFPDNPERWLEYLDDLLYIAKNTQRRNDTDLNTSEDGLNVRLNDRVIESLCDLACLADRLASIIKHPHDAEKASLQDLLYSLSDGELKFTYHSIAENRGVLTNVLNNAVMEAHQELDYQPLLYLPTGVVYIAPKNAPEVSLETLPNRVVDTIKSLCSGELQRKQTGFGRDGKGMKYADYYSQFFDDAGLMRAALNATLRILGDNKASVARSRGENLIKFQQQGVLPTDYDFHCEDDIRIDRLAEFGDVVTRKIWGDRLEKIEQARKLQKNLPAPPDLDLISEIAHYWNLENYLPQIRAIKRINESLKELKLKGNTGGVPYEWYYLAAQYLKQHPGIEDIRPVAEDLIAFLAAKIAAIVAGYNLPDGWEDLREWVNQVVQLPGRELAHSIETFQKELNHYNAAKKQGRGRQLLCSISHSPYSVSEQMESAVLFTPQVYTNKQMLAGSNAKRNISSIAGTEMMLRQILMNQTQAVGKRFEDGKYRYLYFYPTYYFTPETNSFLQKAYANIAQTRFDSSIKLHFVDKNLVANFDRTRYQSVDSFLIDEKLRQKKETINEEEDGKKDRTFKLSYPEDKPLTFYFMALPPGRNPTDTESWVMPAWLGLAFPMILDVKTVVSESPIPPYRDGAEFEETVFLDSAPQAIRSLTRCDRFRLDRVLNPWQDNDGKKYSAPLNTLTAAYSIHLDVNSKQGKTGYDPNWGKLTELAINLETSPLYVFHYFKQWKRGKDADIPSANRIALYLYDFYPCFDPYVQANRTNLTIDMTAESPLNHPKNLTELYRQFYRAKSSKGKPIKANAILKPIDEAADIILKADKAISDDLTSLVAARLFKLMDRVRSQTAEGRYVIKERDQEREKILDFAKYFVKNVFEESFESDRARLAGRQLNIIRDTCEFLYRLEMDKERRQRQVQPLDTSNSSSEEEE

SEQ ID NO: 6 - protein, 160 aa, Microcystis aeruginosa
MTAESPLNHPKNLTELYRQFYRAKSSKGKPIKANAILKPIDEAADIILKADKAISDDLTSLVAARLFKLMDRVRSQTAEGRYVIKERDQEREKILDFAKYFVKNVFEESFESDRARLAGRQLNIIRDTCEFLYRLEMDKERRQRQVQPLDTSNSSSEEEE

SEQ ID NO: 7 - RNA, 109 nt, Artificial
  TiDcrRNA
  misc_feature (38)..(72): n is a, c, g, or u
guuccaauuaaucuuaagcccuauuagggauugaaacnnnnnnnnnnnnnnnnnnnnnnnnnnnnnnnnnnnguuccaauuaaucuuaagcccuauuagggauugaaac

SEQ ID NO: 8 - protein, 153 aa, Anabaena cylindrica
VGEVSTLNHPKKLTELYRRFYRANKRFNPKANAVLKPIDIAAETILKADSSVFDGETLISAVAAEVFKLMDRVHSSTAEGRWIMSKREEERQAVLEFANYFVVEVFEGCFKSDRARLAGRQLNLIRDTCEFLYRLEDDKENAEKSKSEIDENE

SEQ ID NO: 9 - protein, 155 aa, Calothrix PCC6303 (Calothrix parietina)
MPESQLNHPKKLTDLYRKFYRANKRYNPKSNAVLKPIDIAAETILKAEVSVFSGETLVAAVAAEVFKLMDRVHANTADGRWVMSKREEERQAVLDFARYFVMDVFENSFSSDRARLAGRQLNLIKDTCEFLYRLEDDKENANKDVKEEENDKNED

SEQ ID NO: 10 - protein, 139 aa, Crinalium epipsammum
MQMIRDIVDKYACFYRASGFAAYARLRPLNVAMKVVLDSLPHTSKDDLKLMIEGHLIALVDGVLDKQTDGYIPEEVKKDIAQRQEAIETFSGSFLEQVFYDYCKGERSLLRQHINLIRKGSEAYYVKTYSKKKNQQETK

SEQ ID NO: 11 - protein, 152 aa, Cyanothece PCC7424 (Gloeothece citriformis)
MTEKLKKTKDLVNYSRTFYQVKLSDSSHSILLPISKALEIILSTPENIDNEDLIFQGAGQLHDALDRQEVYKRPLLQNKSIPYETRKNQELEAIYQFMRFCVEEVFCQMYKGDKALLQENRNRIKSGAEFAYRWLTLEEQKQEQVTSESIDS

SEQ ID NO: 12 - protein, 162 aa, Gloeobacter kilaueensis
VPETSPLNRPKTLTELYRRFYRAEKRYNASSRSVLRPLDDAASVVMLADPALRSDELVVLVAGGVGKLMDRVRASTAEGRWVIRDREAERLAILEFARYFVEDVFVKTFDSDRARLDGRQLNLLRDACEFLYRLEEDRELAAKPQPPGPDEPASPDESAPAA

SEQ ID NO: 13 - protein, 165 aa, Gloeocapsa sp. PCC7428
VNQLRQLTQLFRRFYRAKSQYAKANAILKPIDEAANVILKFDKTLANDNQCLTDVVYARVAKLMNNVRRGAAEGKPTLKLVDGKWKPALTPEEERQAVYAFAEYFVNEIFEGSFKGDRARLAGTQLNLIRDTCEYLYRLEDDKERQERKVVEPDEISDIENSEVA

SEQ ID NO: 14 - protein, 145 aa, Halothece PCC7418
VNDTKSPMNHPKELTRLFRRFYRANKMYNPKANAILKPIEVASDTILKADNSVFTGETLVAVVAAEVNKLMDRVRASTAEGRWVISQREKERQAVLDFARYFVEEVFEKSFSRDRARLAGRQLNLLKDTCEFLYRLEQDKENSDQ

SEQ ID NO: 15 - protein, 148 aa, Methanospirillum hungatei
MAVASIHELARLGLSVAIPRNYDPHKVEKLFRESVKAILGKRGSQYPREDYVDAVSGRLLKMIKRAGDDQFSRTPGLYDFSLIVSFAEYFVDHIFYQVASGDPGKLKRAANDLADGFYSATLQLREEYFESRKEAFESEQDLSSEQEN

SEQ ID NO: 16 - protein, 148 aa, Nostoc sp. NIES-2111
MTDKLNLINRLVEEYRQFYQVNVGESSHAVLLPLSKALEVILTVPEQIEREDIILQAAGQLNDAIERQEAYKRPFLMDKSVDISTRKAQELAAIHKFMTTCVDDLFMGLYLGDRALLQENRNRIKSGAEFAYRWLALQEKTQLQGEKK

SEQ ID NO: 17 - protein, 162 aa, Rivularia sp. PCC7116
VESESSLCHTQKLTELYRRFYRANKKYNPKSNAVLKPIDIAAETILKAELSVHTGECLVLVVAAEVFKLMDRVHASTAEGRWVFNHKEREEERQAVLEFARYFVEDIFEKSFAGDRARLAGRQINLIRDTCEFLYRLENDKENQLQGNDSKKENDSETLISS

SEQ ID NO: 18 - protein, 158 aa, Stanieria cyanosphaera
MEKLAKSPLNHPLQLTELYRKFYRANKLYNPKANAVLKPIEIAADTILKAESTVFHGETLVHAVAAEVTKLMDRVHASTADGRWVFTNQERDKERQAILEFSRYFVEEVFEKSFAGDRARLAGKQINLIRDTCEFLYRLENDKDIEEKKKNNPDDSEE

SEQ ID NO: 19 - protein, 146 aa, Synechocystis sp. PCC6803
MTEKLKLTKRLVEEYRRFYQVELSKKPSTHAILLPLSKALEQILSVPDDWDEEELILQGSGQLQAALDRQEVYTRPIIKDKSVAYETRQLQELEAIQIFMTTCVRDLFGEMCKGDRAILQEQRNRIKSGAEFAYRLLALEAQQNQN

SEQ ID NO: 20 - DNA, 35 bp, Homo sapiens
cctagtggccccactgtggggtggaggggacagat

SEQ ID NO: 21 - protein, 6 aa, Artificial
  NLS
KKKKRK

SEQ ID NO: 22 - DNA, 105 bp, Artificial
  DNA fragment for pre-mature crRNA
gttccaattaatcttaagccctattagggattgaaacggagaccctcaattgtcggtctcgttccaattaatcttaagccctattagggattgaaactttttttt

SEQ ID NO: 23 - DNA, 30 bp, Homo sapiens
cctagtggccccactgtggggtggagggga

SEQ ID NO: 24 - DNA, 30 bp, Artificial
  Primer F1
cttagcataatgtcctcaagatacatctac

SEQ ID NO: 25 - DNA, 30 bp, Artificial
  Primer R1
gatatgtaaccattattctagatggctatg

SEQ ID NO: 26 - DNA, 28 bp, Artificial
  Primer F2
gggtccaagggaaaaggaggactgatcc

SEQ ID NO: 27 - DNA, 30 bp, Artificial
  Primer R2
ataaacacaaactcataaacaacatacatc

SEQ ID NO: 28 - DNA, 35 bp, Artificial
  Nonspecific sequence
aaataaatagcggtcgggtgccccgaatttcacat

SEQ ID NO: 29 - protein, 160 aa, Escherichia coli
MADEIDAMALYRAWQQLDNGSCAQIRRVSEPDELRDIPAFYRLVQPFGWENPRHQQALLRMVFCLSAGKNVIRHQDKKSEQTTGISLGRALANSGRINERRIFQLIRADRTADMVQLRRLLTHAEPVLDWPLMARMLTWWGKRERQQLLEDFVLTTNKNA

SEQ ID NO: 30 - protein, 186 aa, Acetobacter pasteurianus
MLLSNKEAIRQVVNWWHGLQPDPERKQFGDRATLARLRRCATVTEALFEPQTQALVHKCGAKKDSELSRLALVAAVLAHVRANKTGACMARLIGPSDTSDSATALCKPVRFRRLLDMETYDDCLRSFRRLVVMAGEPLDVADLARSVIMWPREDTWDDLAGDQVRRQWVYNYWNAGIPENSSEKHN

SEQ ID NO: 31 - protein, 190 aa, Acidimicrobium ferrooxidans
MTTTSSTSTNDTLFRQVRDMIARDPGALATLRRNVGRSFDESPDSWPYVLMVTGRSRWREPAAHLALGLFALHHQSKTPGALDKEGSTFGLATRRLRTSRGDSGASEQGIERRFRSALASETIDALGVHLRGLVTLMRGADVSLDYPRLYQDLSTWLLPEKLQRVSLRWARDYYALDPDQQSPAEQKEEP

SEQ ID NO: 32 - protein, 198 aa, Amycolatopsis mediterranei
MSTPVAQRRDGFISALYALNAGLESSIPKRRSEARQVLARLRRSLVTARPEPAAYEVVFRHDPPESEQDAWILVAGLFALHPKASRRGDRSIGTAMQALQDKRGDSATRRFEQLLGRDRAGLPHHLRQIVRLLAAEGIPVNYAALLDDLVVLMGDKYSEDTAHRIRLRWARDFHRKRKTTTTDNGEPAPAPTTVENPA

SEQ ID NO: 33 - protein, 222 aa, Bifidobacterium animalis
MMNENSDEGKIRLSPFGQWVARKAAMLATGGGSDKATAGGYIGNDSKAVAAIAQLAHAAGHEVGADPDIFVWTVPDEDDAAIYPYRVPHDCAPTAEEMAAHLAMTLFAVQQQSHREQSMQTDSNMSLGRAVGMIAYGNFNEKGIRSTFDKMQTANGWAEMSHHARRLIKLLKREEIPLNYGLLAQDLVRLRRGRETANLVRLQWGRDYQSGYRAAMNAASDE

SEQ ID NO: 34 - protein, 216 aa, Cellulomonas fimi
MTETRTPPVDDDLEESTTPPRTTREFVSWQVGRLQREYLPPVQSSWARASLAELRRSLTQPLGSSPAVLEFVVNPSAPTTDGPETPDERSIVTALGLYAVHQQSQSVPMHLRSVGFGDAVGRIRLRDGDEVRGVTRRFQALGTAQTWDELVHHARGLVQLLRDRQQGFDYGRFAEDLVQFQHPASADRVRLRWGRAFYRVTTAPTTSTSTTTAEEQ

SEQ ID NO: 35 - protein, 219 aa, Coriobacterium glomerans
MSNTYEVAGKLGAFAARKIQILQRDYLGSGSRAAHARSVLAQLRRLHEPGSSTWIMAGRELFENWPELDLGPSEETRALRAVATSFKFYAIHQQSNTVGMSMPHKKKDGAQVPRRNPYSFGQACRQIDPDIDRSGAIRRRLASIEAAYDFEGIAYHMRGLIKLMSSKQIGLDYFSLIKDLYLVQCDGLKDRVLIDWSRAYFGSLETEPQKAAAIEIEKA

SEQ ID NO: 36 - protein, 171 aa, Cyanothece (Gloeothece citriformis) PCC7424
MTTTEISKERAFINAVWQRIEGNRGAIATVSRCTDSDPYYQRQAATYIYPYLPDDIRQWQKKINRYVFVAALMAKNHQQNPKDAQIGSSFGHTCLRLKKHANVNANGIENRFQALLNANGEDVYRYLGMFAPLLRQHNIPCEWAKLLEDLNCWDHEEEKVRLRWARDFYQD

SEQ ID NO: 37 - protein, 192 aa, Desulfococcus oleovorans
MSEYYYLDAESCQLLQRWHHWLDNNRGDRARLRRAERPEDVLLTEAFFNFLKQMPNSWQEQKPIFSSAAVAGLLSHVKADHQVVSKGYQPKDEKKSKKMASFSEQLATSIKGDRGAMSELRFQQLQKSRTTDEFYRRMVRAIRLLDGRVNILSLANDIIQWHKEHDREFDRKPANRLAVRWATDYFSVLPNN

SEQ ID NO: 38 - protein, 156 aa, Erwinia amylovora
MELPSDAKALYENWLQLDPGSKAKIRRATQPDDLMDIPAFYLLVAPFGWPQQRYALLRMVFCLSAGKIRPSEDKQQSIGRVFADKGISQPRIFQVIRADYPNDMVQLRRLIIHAEPEVYWPGFAQQLYGWYKSDRRKLLEDFVITTAHKTSRKDAK

SEQ ID NO: 39 - protein, 158 aa, Frankia alni
MRRGVGREPGSVPQMWRYYTTLQADGHLTTRLRAEHAALTLFAIHQQSLPRSAHELGSGLGTAVKELRASGKFSPDAVDRRFGTAATATSLSEASYHLRGLVRQLRQIQRPLDYTALFWDLVTWQNPARLGQVRRRWAAQYFLNRDSEGAASASASRR

SEQ ID NO: 40 - protein, 147 aa, Geobacter sulfurreducens
MERTHDFMGLYQAWERLAPGPRAELRRVERPDDLLEVPAFYRLFSGRGTTEWEKGAYQRLIFCLPCIKHSGENISLGRALAKGRGVGEKRLFQVVRSSEPNDMIQLRRILRMAEPTVNWDLAARQLWYWNDRSKRDLLEDYFLNHSN

SEQ ID NO: 41 - protein, 200 aa, Kitasatospora setae
MTTDQPTARRRYWDEYTAPDHGWRIDGPSKQPRRPPGEELAALRSGLGRPVMDSPKMWPYYSTEVGDVLALRDRVSDEQQAEHAALALYGLHQQGQSRPMHRSGVKLGRALRELRRDGKYSENALDARVAQLAAATSVPALLVHLRGLVTQLRTVGQPLDYDHLMADIRAWHQSERRPQVRLKWALGYRAWQSKTPDDDE

SEQ ID NO: 42 - protein, 194 aa, Lactobacillus fermentum
MSHISKTVAKIIHQLYNDGDLDKGTLAKLRTANSLLSRDATAIWPLLFENIEDKQDLSQTGEPSFAETAIFTALRAYAIYQQGTEESVFKHSDNWRENRSLFQAFGRLRSDPDFTDSLDKRVSNVLTSLNFQSAENSITQLVRILKSKGQGGQIDFAQLGEDLYRFQFSSESARQVTLKWGQDYYWNNLKDNQE